European Patent Application EP 4 335 932 A2, published March 13, 2024. Title: METHODS OF MONITORING CONDITIONS BY SEQUENCE ANALYSIS. Applicant: ADAPTIVE BIOTECHNOLOGIES CORPORATION. Application EP 24152841.3, filed January 19, 2024. The sequence listing filed with the application follows.

SEQUENCE LISTING (135 sequences)

SEQ ID NO: 1 - DNA, 23 bp, synthetic construct
  misc_feature 1..23: note = source = /note="Description of Artificial Sequence: Synthetic primer"
  source 1..23: mol_type = other DNA
aactatgttttggtatcgtcagt

SEQ ID NO: 2 - DNA, 19 bp, synthetic construct
  misc_feature 1..19: note = source = /note="Description of Artificial Sequence: Synthetic primer"
  source 1..19: mol_type = other DNA
ttctggtaccgtcagcaac

SEQ ID NO: 3 - DNA, 21 bp, synthetic construct
  misc_feature 1..21: note = source = /note="Description of Artificial Sequence: Synthetic primer"
  source 1..21: mol_type = other DNA
agtgtatcctggtaccaacag

SEQ ID NO: 4 - DNA, 21 bp, synthetic construct
  misc_feature 1..21: note = source = /note="Description of Artificial Sequence: Synthetic primer"
  source 1..21: mol_type = other DNA
agtgtgtactggtaccaacag

SEQ ID NO: 5 - DNA, 21 bp, synthetic construct
  misc_feature 1..21: note = source = /note="Description of Artificial Sequence: Synthetic primer"
  source 1..21: mol_type = other DNA
actgtgtcctggtaccaacag

SEQ ID NO: 6 - DNA, 21 bp, synthetic construct
  misc_feature 1..21: note = source = /note="Description of Artificial Sequence: Synthetic primer"
  source 1..21: mol_type = other DNA
agtgtgtcctggtaccaacag

SEQ ID NO: 7 - DNA, 21 bp, synthetic construct
  misc_feature 1..21: note = source = /note="Description of Artificial Sequence: Synthetic primer"
  source 1..21: mol_type = other DNA
tctgtgtactggtaccaacag

SEQ ID NO: 8 - DNA, 20 bp, synthetic construct
  misc_feature 1..20: note = source = /note="Description of Artificial Sequence: Synthetic primer"
  source 1..20: mol_type = other DNA
ccctttactggtaccgacag

SEQ ID NO: 9 - DNA, 20 bp, synthetic construct
  misc_feature 1..20: note = source = /note="Description of Artificial Sequence: Synthetic primer"
  source 1..20: mol_type = other DNA
gcctttactggtaccgacag

SEQ ID NO: 10 - DNA, 21 bp, synthetic construct
  misc_feature 1..21: note = source = /note="Description of Artificial Sequence: Synthetic primer"
  source 1..21: mol_type = other DNA
ccctttactggtaccgacaaa

SEQ ID NO: 11 - DNA, 19 bp, synthetic construct
  misc_feature 1..19: note = source = /note="Description of Artificial Sequence: Synthetic primer"
  source 1..19: mol_type = other DNA
ttttggtaccaacaggtcc

SEQ ID NO: 12 - DNA, 19 bp, synthetic construct
  misc_feature 1..19: note = source = /note="Description of Artificial Sequence: Synthetic primer"
  source 1..19: mol_type = other DNA
ttttggtaccaacaggccc

SEQ ID NO: 13 - DNA, 22 bp, synthetic construct
  misc_feature 1..22: note = source = /note="Description of Artificial Sequence: Synthetic primer"
  source 1..22: mol_type = other DNA
aaccctttattggtatcaacag

SEQ ID NO: 14 - DNA, 21 bp, synthetic construct
  misc_feature 1..21: note = source = /note="Description of Artificial Sequence: Synthetic primer"
  source 1..21: mol_type = other DNA
cgctatgtattggtacaagca

SEQ ID NO: 15 - DNA, 21 bp, synthetic construct
  misc_feature 1..21: note = source = /note="Description of Artificial Sequence: Synthetic primer"
  source 1..21: mol_type = other DNA
ggcaatgtattggtacaagca

SEQ ID NO: 16 - DNA, 23 bp, synthetic construct
  misc_feature 1..23: note = source = /note="Description of Artificial Sequence: Synthetic primer"
  source 1..23: mol_type = other DNA
tttctggtacagacagaccatga

SEQ ID NO: 17 - DNA, 27 bp, synthetic construct
  misc_feature 1..27: note = source = /note="Description of Artificial Sequence: Synthetic primer"
  source 1..27: mol_type = other DNA
tactatgtattggtataaacaggactc

SEQ ID NO: 18 - DNA, 22 bp, synthetic construct
  misc_feature 1..22: note = source = /note="Description of Artificial Sequence: Synthetic primer"
  source 1..22: mol_type = other DNA
caaaatgtactggtatcaacaa

SEQ ID NO: 19 - DNA, 22 bp, synthetic construct
  misc_feature 1..22: note = source = /note="Description of Artificial Sequence: Synthetic primer"
  source 1..22: mol_type = other DNA
atgttctggtatcgacaagacc

SEQ ID NO: 20 - DNA, 22 bp, synthetic construct
  misc_feature 1..22: note = source = /note="Description of Artificial Sequence: Synthetic primer"
  source 1..22: mol_type = other DNA
atgtactggtatcgacaagacc

SEQ ID NO: 21 - DNA, 23 bp, synthetic construct
  misc_feature 1..23: note = source = /note="Description of Artificial Sequence: Synthetic primer"
  source 1..23: mol_type = other DNA
tgccatgtactggtatagacaag

SEQ ID NO: 22 - DNA, 23 bp, synthetic construct
  misc_feature 1..23: note = source = /note="Description of Artificial Sequence: Synthetic primer"
  source 1..23: mol_type = other DNA
atacttgtcctggtatcgacaag

SEQ ID NO: 23 - DNA, 22 bp, synthetic construct
  misc_feature 1..22: note = source = /note="Description of Artificial Sequence: Synthetic primer"
  source 1..22: mol_type = other DNA
atatgttctggtatcgacaaga

SEQ ID NO: 24 - DNA, 22 bp, synthetic construct
  misc_feature 1..22: note = source = /note="Description of Artificial Sequence: Synthetic primer"
  source 1..22: mol_type = other DNA
atatgtcctggtatcgacaaga

SEQ ID NO: 25 - DNA, 22 bp, synthetic construct
  misc_feature 1..22: note = source = /note="Description of Artificial Sequence: Synthetic primer"
  source 1..22: mol_type = other DNA
acatgtcctggtatcgacaaga

SEQ ID NO: 26 - DNA, 24 bp, synthetic construct
  misc_feature 1..24: note = source = /note="Description of Artificial Sequence: Synthetic primer"
  source 1..24: mol_type = other DNA
taatctttattggtatcgacgtgt

SEQ ID NO: 27 - DNA, 20 bp, synthetic construct
  misc_feature 1..20: note = source = /note="Description of Artificial Sequence: Synthetic primer"
  source 1..20: mol_type = other DNA
gccatgtactggtaccgaca

SEQ ID NO: 28 - DNA, 22 bp, synthetic construct
  misc_feature 1..22: note = source = /note="Description of Artificial Sequence: Synthetic primer"
  source 1..22: mol_type = other DNA
tcatgtttactggtatcggcag

SEQ ID NO: 29 - DNA, 21 bp, synthetic construct
  misc_feature 1..21: note = source = /note="Description of Artificial Sequence: Synthetic primer"
  source 1..21: mol_type = other DNA
caacctatactggtaccgaca

SEQ ID NO: 30 - DNA, 22 bp, synthetic construct
  misc_feature 1..22: note = source = /note="Description of Artificial Sequence: Synthetic primer"
  source 1..22: mol_type = other DNA
catgctaccctttactggtacc

SEQ ID NO: 31 - DNA, 22 bp, synthetic construct
  misc_feature 1..22: note = source = /note="Description of Artificial Sequence: Synthetic primer"
  source 1..22: mol_type = other DNA
cacaataccctttactggtacc

SEQ ID NO: 32 - DNA, 26 bp, synthetic construct
  misc_feature 1..26: note = source = /note="Description of Artificial Sequence: Synthetic primer"
  source 1..26: mol_type = other DNA
atacttctattggtacagacaaatct

SEQ ID NO: 33 - DNA, 21 bp, synthetic construct
  misc_feature 1..21: note = source = /note="Description of Artificial Sequence: Synthetic primer"
  source 1..21: mol_type = other DNA
cactgtctactggtaccagca

SEQ ID NO: 34 - DNA, 21 bp, synthetic construct
  misc_feature 1..21: note = source = /note="Description of Artificial Sequence: Synthetic primer"
  source 1..21: mol_type = other DNA
cgtcatgtactggtaccagca

SEQ ID NO: 35 - DNA, 21 bp, synthetic construct
  misc_feature 1..21: note = source = /note="Description of Artificial Sequence: Synthetic primer"
  source 1..21: mol_type = other DNA
aatgatacggcgaccaccgag

SEQ ID NO: 36 - DNA, 24 bp, synthetic construct
  misc_feature 1..24: note = source = /note="Description of Artificial Sequence: Synthetic primer"
  source 1..24: mol_type = other DNA
caagcagaagacggcatacgagat

SEQ ID NO: 37 - DNA, 34 bp, synthetic construct
  misc_feature 1..34: note = source = /note="Description of Artificial Sequence: Synthetic primer"
  source 1..34: mol_type = other DNA
agatcggaagagcacacgtctgaactccagtcac

SEQ ID NO: 38 - DNA, 34 bp, synthetic construct
  misc_feature 1..34: note = source = /note="Description of Artificial Sequence: Synthetic primer"
  source 1..34: mol_type = other DNA
gtgactggagttcagacgtgtgctcttccgatct

SEQ ID NO: 39 - DNA, 24 bp, synthetic construct
  misc_feature 1..24: note = source = /note="Description of Artificial Sequence: Synthetic primer"
  source 1..24: mol_type = other DNA
cctcagtgaaggtctcctgcaagg

SEQ ID NO: 40 - DNA, 24 bp, synthetic construct
  misc_feature 1..24: note = source = /note="Description of Artificial Sequence: Synthetic primer"
  source 1..24: mol_type = other DNA
cctcggtgaaggtctcctgcaagg

SEQ ID NO: 41 - DNA, 24 bp, synthetic construct
  misc_feature 1..24: note = source = /note="Description of Artificial Sequence: Synthetic primer"
  source 1..24: mol_type = other DNA
cctcagtgaaggtttcctgcaagg

SEQ ID NO: 42 - DNA, 27 bp, synthetic construct
  misc_feature 1..27: note = source = /note="Description of Artificial Sequence: Synthetic primer"
  source 1..27: mol_type = other DNA
gggctacagtgaaaatctcctgcaagg

SEQ ID NO: 43 - DNA, 26 bp, synthetic construct
  misc_feature 1..26: note = source = /note="Description of Artificial Sequence: Synthetic primer"
  source 1..26: mol_type = other DNA
aaacccacacagaccctcacgctgac

SEQ ID NO: 44 - DNA, 26 bp, synthetic construct
  misc_feature 1..26: note = source = /note="Description of Artificial Sequence: Synthetic primer"
  source 1..26: mol_type = other DNA
aaacccacagagaccctcacgctgac

SEQ ID NO: 45 - DNA, 26 bp, synthetic construct
  misc_feature 1..26: note = source = /note="Description of Artificial Sequence: Synthetic primer"
  source 1..26: mol_type = other DNA
aaacccacacagaccctcacactgac

SEQ ID NO: 46 - DNA, 25 bp, synthetic construct
  misc_feature 1..25: note = source = /note="Description of Artificial Sequence: Synthetic primer"
  source 1..25: mol_type = other DNA
ctggggggtccctgagactctcctg

SEQ ID NO: 47 - DNA, 25 bp, synthetic construct
  misc_feature 1..25: note = source = /note="Description of Artificial Sequence: Synthetic primer"
  source 1..25: mol_type = other DNA
ctggggggtcccttagactctcctg

SEQ ID NO: 48 - DNA, 25 bp, synthetic construct
  misc_feature 1..25: note = source = /note="Description of Artificial Sequence: Synthetic primer"
  source 1..25: mol_type = other DNA
cagggcggtccctgagactctcctg

SEQ ID NO: 49 - DNA, 25 bp, synthetic construct
  misc_feature 1..25: note = source = /note="Description of Artificial Sequence: Synthetic primer"
  source 1..25: mol_type = other DNA
cagggccgtccctgagactctcctg

SEQ ID NO: 50 - DNA, 25 bp, synthetic construct
  misc_feature 1..25: note = source = /note="Description of Artificial Sequence: Synthetic primer"
  source 1..25: mol_type = other DNA
ctggggggtccctgaaactctcctg

SEQ ID NO: 51 - DNA, 25 bp, synthetic construct
  misc_feature 1..25: note = source = /note="Description of Artificial Sequence: Synthetic primer"
  source 1..25: mol_type = other DNA
ctggcaggtccctgagactctcctg

SEQ ID NO: 52 - DNA, 25 bp, synthetic construct
  misc_feature 1..25: note = source = /note="Description of Artificial Sequence: Synthetic primer"
  source 1..25: mol_type = other DNA
ctggagggtccctgagactctcctg

SEQ ID NO: 53 - DNA, 25 bp, synthetic construct
  misc_feature 1..25: note = source = /note="Description of Artificial Sequence: Synthetic primer"
  source 1..25: mol_type = other DNA
ctgggaggtccctgagactctcctg

SEQ ID NO: 54 - DNA, 23 bp, synthetic construct
  misc_feature 1..23: note = source = /note="Description of Artificial Sequence: Synthetic primer"
  source 1..23: mol_type = other DNA
tgggggggccctgagactctcct

SEQ ID NO: 55 - DNA, 25 bp, synthetic construct
  misc_feature 1..25: note = source = /note="Description of Artificial Sequence: Synthetic primer"
  source 1..25: mol_type = other DNA
cttcggagaccctgtccctcacctg

SEQ ID NO: 56 - DNA, 25 bp, synthetic construct
  misc_feature 1..25: note = source = /note="Description of Artificial Sequence: Synthetic primer"
  source 1..25: mol_type = other DNA
cttcggacaccctgtccctcacctg

SEQ ID NO: 57 - DNA, 25 bp, synthetic construct
  misc_feature 1..25: note = source = /note="Description of Artificial Sequence: Synthetic primer"
  source 1..25: mol_type = other DNA
cttcacagaccctgtccctcacctg

SEQ ID NO: 58 - DNA, 25 bp, synthetic construct
  misc_feature 1..25: note = source = /note="Description of Artificial Sequence: Synthetic primer"
  source 1..25: mol_type = other DNA
cttcggagaccccgtccctcacctg

SEQ ID NO: 59 - DNA, 22 bp, synthetic construct
  misc_feature 1..22: note = source = /note="Description of Artificial Sequence: Synthetic primer"
  source 1..22: mol_type = other DNA
cggggaccctgtccctcacctg

SEQ ID NO: 60 - DNA, 29 bp, synthetic construct
  misc_feature 1..29: note = source = /note="Description of Artificial Sequence: Synthetic primer"
  source 1..29: mol_type = other DNA
gatctcctgtaagggttctggatacagct

SEQ ID NO: 61 - DNA, 25 bp, synthetic construct
  misc_feature 1..25: note = source = /note="Description of Artificial Sequence: Synthetic primer"
  source 1..25: mol_type = other DNA
tcgcagaccctctcactcacctgtg

SEQ ID NO: 62 - DNA, 25 bp, synthetic construct
  misc_feature 1..25: note = source = /note="Description of Artificial Sequence: Synthetic primer"
  source 1..25: mol_type = other DNA
tggatcaggcagtccccatcgagag

SEQ ID NO: 63 - DNA, 20 bp, synthetic construct
  misc_feature 1..20: note = source = /note="Description of Artificial Sequence: Synthetic primer"
  source 1..20: mol_type = other DNA
gctgggtgcgccagatgccc

SEQ ID NO: 64 - DNA, 20 bp, synthetic construct
  misc_feature 1..20: note = source = /note="Description of Artificial Sequence: Synthetic primer"
  source 1..20: mol_type = other DNA
tggatccgtcagcccccagg

SEQ ID NO: 65 - DNA, 20 bp, synthetic construct
  misc_feature 1..20: note = source = /note="Description of Artificial Sequence: Synthetic primer"
  source 1..20: mol_type = other DNA
tggatccgtcagcccccggg

SEQ ID NO: 66 - DNA, 21 bp, synthetic construct
  misc_feature 1..21: note = source = /note="Description of Artificial Sequence: Synthetic primer"
  source 1..21: mol_type = other DNA
gtgcgacaggcccctggacaa

SEQ ID NO: 67 - DNA, 23 bp, synthetic construct
  misc_feature 1..23: note = source = /note="Description of Artificial Sequence: Synthetic primer"
  source 1..23: mol_type = other DNA
gggtgcgacaggccactggacaa

SEQ ID NO: 68 - DNA, 21 bp, synthetic construct
  misc_feature 1..21: note = source = /note="Description of Artificial Sequence: Synthetic primer"
  source 1..21: mol_type = other DNA
gtgcgccaggcccccggacaa

SEQ ID NO: 69 - DNA, 23 bp, synthetic construct
  misc_feature 1..23: note = source = /note="Description of Artificial Sequence: Synthetic primer"
  source 1..23: mol_type = other DNA
gggtgcgacaggctcgtggacaa

SEQ ID NO: 70 - DNA, 23 bp, synthetic construct
  misc_feature 1..23: note = source = /note="Description of Artificial Sequence: Synthetic primer"
  source 1..23: mol_type = other DNA
gggtgcaacaggcccctggaaaa

SEQ ID NO: 71 - DNA, 23 bp, synthetic construct
  misc_feature 1..23: note = source = /note="Description of Artificial Sequence: Synthetic primer"
  source 1..23: mol_type = other DNA
gggtgcgacaggctcctggaaaa

SEQ ID NO: 72 - DNA, 21 bp, synthetic construct
  misc_feature 1..21: note = source = /note="Description of Artificial Sequence: Synthetic primer"
  source 1..21: mol_type = other DNA
gtgcgacaggcccccggacaa

SEQ ID NO: 73 - DNA, 21 bp, synthetic construct
  misc_feature 1..21: note = source = /note="Description of Artificial Sequence: Synthetic primer"
  source 1..21: mol_type = other DNA
gtgcgacaggcccccagacaa

SEQ ID NO: 74 - DNA, 21 bp, synthetic construct
  misc_feature 1..21: note = source = /note="Description of Artificial Sequence: Synthetic primer"
  source 1..21: mol_type = other DNA
tccgccagcccccagggaagg

SEQ ID NO: 75 - DNA, 21 bp, synthetic construct
  misc_feature 1..21: note = source = /note="Description of Artificial Sequence: Synthetic primer"
  source 1..21: mol_type = other DNA
tccggcagcccccagggaagg

SEQ ID NO: 76 - DNA, 21 bp, synthetic construct
  misc_feature 1..21: note = source = /note="Description of Artificial Sequence: Synthetic primer"
  source 1..21: mol_type = other DNA
tccggcagccaccagggaagg

SEQ ID NO: 77 - DNA, 21 bp, synthetic construct
  misc_feature 1..21: note = source = /note="Description of Artificial Sequence: Synthetic primer"
  source 1..21: mol_type = other DNA
tccgccagcacccagggaagg

SEQ ID NO: 78 - DNA, 19 bp, synthetic construct
  misc_feature 1..19: note = source = /note="Description of Artificial Sequence: Synthetic primer"
  source 1..19: mol_type = other DNA
tccggcagcccgccgggaa

SEQ ID NO: 79 - DNA, 19 bp, synthetic construct
  misc_feature 1..19: note = source = /note="Description of Artificial Sequence: Synthetic primer"
  source 1..19: mol_type = other DNA
tccggcagccgccggggaa

SEQ ID NO: 80 - DNA, 21 bp, synthetic construct
  misc_feature 1..21: note = source = /note="Description of Artificial Sequence: Synthetic primer"
  source 1..21: mol_type = other DNA
tccggcagcccgctgggaagg

SEQ ID NO: 81 - DNA, 21 bp, synthetic construct
  misc_feature 1..21: note = source = /note="Description of Artificial Sequence: Synthetic primer"
  source 1..21: mol_type = other DNA
tccgccagcccctagggaagg

SEQ ID NO: 82 - DNA, 21 bp, synthetic construct
  misc_feature 1..21: note = source = /note="Description of Artificial Sequence: Synthetic primer"
  source 1..21: mol_type = other DNA
ggtccgccaggctccagggaa

SEQ ID NO: 83 - DNA, 21 bp, synthetic construct
  misc_feature 1..21: note = source = /note="Description of Artificial Sequence: Synthetic primer"
  source 1..21: mol_type = other DNA
gttccgccaggctccagggaa

SEQ ID NO: 84 - DNA, 21 bp, synthetic construct
  misc_feature 1..21: note = source = /note="Description of Artificial Sequence: Synthetic primer"
  source 1..21: mol_type = other DNA
ggtccgccaggcttccgggaa

SEQ ID NO: 85 - DNA, 21 bp, synthetic construct
  misc_feature 1..21: note = source = /note="Description of Artificial Sequence: Synthetic primer"
  source 1..21: mol_type = other DNA
ggtccgtcaagctccggggaa

SEQ ID NO: 86 - DNA, 21 bp, synthetic construct
  misc_feature 1..21: note = source = /note="Description of Artificial Sequence: Synthetic primer"
  source 1..21: mol_type = other DNA
gatccgccaggctccagggaa

SEQ ID NO: 87 - DNA, 21 bp, synthetic construct
  misc_feature 1..21: note = source = /note="Description of Artificial Sequence: Synthetic primer"
  source 1..21: mol_type = other DNA
ggtccgccaagctccagggaa

SEQ ID NO: 88 - DNA, 21 bp, synthetic construct
  misc_feature 1..21: note = source = /note="Description of Artificial Sequence: Synthetic primer"
  source 1..21: mol_type = other DNA
ggtccgccaggctccaggcaa

SEQ ID NO: 89 - DNA, 21 bp, synthetic construct
  misc_feature 1..21: note = source = /note="Description of Artificial Sequence: Synthetic primer"
  source 1..21: mol_type = other DNA
ggtccgccaggccccaggcaa

SEQ ID NO: 90 - DNA, 21 bp, synthetic construct
  misc_feature 1..21: note = source = /note="Description of Artificial Sequence: Synthetic primer"
  source 1..21: mol_type = other DNA
ggtccgccaggctccgggcaa

SEQ ID NO: 91 - DNA, 24 bp, synthetic construct
  misc_feature 1..24: note = source = /note="Description of Artificial Sequence: Synthetic primer"
  source 1..24: mol_type = other DNA
gggtccgtcaagctccagggaagg

SEQ ID NO: 92 - DNA, 24 bp, synthetic construct
  misc_feature 1..24: note = source = /note="Description of Artificial Sequence: Synthetic primer"
  source 1..24: mol_type = other DNA
ctgggtccgccaagctacaggaaa

SEQ ID NO: 93 - DNA, 21 bp, synthetic construct
  misc_feature 1..21: note = source = /note="Description of Artificial Sequence: Synthetic primer"
  source 1..21: mol_type = other DNA
ggtccgccagcctccagggaa

SEQ ID NO: 94 - DNA, 21 bp, synthetic construct
  misc_feature 1..21: note = source = /note="Description of Artificial Sequence: Synthetic primer"
  source 1..21: mol_type = other DNA
ggtccggcaagctccagggaa

SEQ ID NO: 95 - DNA, 25 bp, synthetic construct
  misc_feature 1..25: note = source = /note="Description of Artificial Sequence: Synthetic primer"
  source 1..25: mol_type = other DNA
ctaaaggctgaggacactgccgtgt

SEQ ID NO: 96 - DNA, 25 bp, synthetic construct
  misc_feature 1..25: note = source = /note="Description of Artificial Sequence: Synthetic primer"
  source 1..25: mol_type = other DNA
ctctgtgactcccgaggacacggct

SEQ ID NO: 97 - DNA, 22 bp, synthetic construct
  misc_feature 1..22: note = source = /note="Description of Artificial Sequence: Synthetic primer"
  source 1..22: mol_type = other DNA
agtggagcagcctgaaggcctc

SEQ ID NO: 98 - DNA, 25 bp, synthetic construct
  misc_feature 1..25: note = source = /note="Description of Artificial Sequence: Synthetic primer"
  source 1..25: mol_type = other DNA
tgaccaacatggaccctgtggacac

SEQ ID NO: 99 - DNA, 25 bp, synthetic construct
  misc_feature 1..25: note = source = /note="Description of Artificial Sequence: Synthetic primer"
  source 1..25: mol_type = other DNA
acatggagctgagcagcctgagatc

SEQ ID NO: 100 - DNA, 25 bp, synthetic construct
  misc_feature 1..25: note = source = /note="Description of Artificial Sequence: Synthetic primer"
  source 1..25: mol_type = other DNA
acatggagctgagcaggctgagatc

SEQ ID NO: 101 - DNA, 25 bp, synthetic construct
  misc_feature 1..25: note = source = /note="Description of Artificial Sequence: Synthetic primer"
  source 1..25: mol_type = other DNA
acatggagctgaggagcctgagatc

SEQ ID NO: 102 - DNA, 28 bp, synthetic construct
  misc_feature 1..28: note = source = /note="Description of Artificial Sequence: Synthetic primer"
  source 1..28: mol_type = other DNA
acatggagctgaggagcctaagatctga

SEQ ID NO: 103 - DNA, 22 bp, synthetic construct
  misc_feature 1..22: note = source = /note="Description of Artificial Sequence: Synthetic primer"
  source 1..22: mol_type = other DNA
gagctctgtgaccgccgcggac

SEQ ID NO: 104 - DNA, 23 bp, synthetic construct
  misc_feature 1..23: note = source = /note="Description of Artificial Sequence: Synthetic primer"
  source 1..23: mol_type = other DNA
gagctctgtgaccgccgtggaca

SEQ ID NO: 105 - DNA, 25 bp, synthetic construct
  misc_feature 1..25: note = source = /note="Description of Artificial Sequence: Synthetic primer"
  source 1..25: mol_type = other DNA
gagctctgtgaccgctgcagacacg

SEQ ID NO: 106 - DNA, 23 bp, synthetic construct
  misc_feature 1..23: note = source = /note="Description of Artificial Sequence: Synthetic primer"
  source 1..23: mol_type = other DNA
gagctctgtgaccgctgcggaca

SEQ ID NO: 107 - DNA, 25 bp, synthetic construct
  misc_feature 1..25: note = source = /note="Description of Artificial Sequence: Synthetic primer"
  source 1..25: mol_type = other DNA
gagctctgtgactgccgcagacacg

SEQ ID NO: 108 - DNA, 25 bp, synthetic construct
  misc_feature 1..25: note = source = /note="Description of Artificial Sequence: Synthetic primer"
  source 1..25: mol_type = other DNA
gagctctgtgactgcagcagacacg

SEQ ID NO: 109 - DNA, 23 bp, synthetic construct
  misc_feature 1..23: note = source = /note="Description of Artificial Sequence: Synthetic primer"
  source 1..23: mol_type = other DNA
gagctctgtgactgccgcggaca

SEQ ID NO: 110 - DNA, 22 bp, synthetic construct
  misc_feature 1..22: note = source = /note="Description of Artificial Sequence: Synthetic primer"
  source 1..22: mol_type = other DNA
gagctctgtgaccgcggacgcg

SEQ ID NO: 111 - DNA, 21 bp, synthetic construct
  misc_feature 1..21: note = source = /note="Description of Artificial Sequence: Synthetic primer"
  source 1..21: mol_type = other DNA
ggctctgtgaccgccgcggac

SEQ ID NO: 112 - DNA, 23 bp, synthetic construct
  misc_feature 1..23: note = source = /note="Description of Artificial Sequence: Synthetic primer"
  source 1..23: mol_type = other DNA
gagctctgtgaccgccgcagaca

SEQ ID NO: 113 - DNA, 23 bp, synthetic construct
  misc_feature 1..23: note = source = /note="Description of Artificial Sequence: Synthetic primer"
  source 1..23: mol_type = other DNA
gagctctgtgaccgctgacacgg

SEQ ID NO: 114 - DNA, 28 bp, synthetic construct
  misc_feature 1..28: note = source = /note="Description of Artificial Sequence: Synthetic primer"
  source 1..28: mol_type = other DNA
caaatgaacagcctgagagccgaggaca

SEQ ID NO: 115 - DNA, 28 bp, synthetic construct
  misc_feature 1..28: note = source = /note="Description of Artificial Sequence: Synthetic primer"
  source 1..28: mol_type = other DNA
caaatgaacagcctgaaaaccgaggaca

SEQ ID NO: 116 - DNA, 28 bp, synthetic construct
  misc_feature 1..28: note = source = /note="Description of Artificial Sequence: Synthetic primer"
  source 1..28: mol_type = other DNA
caaatgaacagtctgaaaaccgaggaca

SEQ ID NO: 117 - DNA, 28 bp, synthetic construct
  misc_feature 1..28: note = source = /note="Description of Artificial Sequence: Synthetic primer"
  source 1..28: mol_type = other DNA
caaatgatcagcctgaaaaccgaggaca

SEQ ID NO: 118 - DNA, 30 bp, synthetic construct
  misc_feature 1..30: note = source = /note="Description of Artificial Sequence: Synthetic primer"
  source 1..30: mol_type = other DNA
caaatgaacagtctgagaactgaggacacc

SEQ ID NO: 119 - DNA, 28 bp, synthetic construct
  misc_feature 1..28: note = source = /note="Description of Artificial Sequence: Synthetic primer"
  source 1..28: mol_type = other DNA
caaatgaacagtctgagagccgaggaca

SEQ ID NO: 120 - DNA, 28 bp, synthetic construct
  misc_feature 1..28: note = source = /note="Description of Artificial Sequence: Synthetic primer"
  source 1..28: mol_type = other DNA
caaatgaacagcctgagagctgaggaca

SEQ ID NO: 121 - DNA, 28 bp, synthetic construct
  misc_feature 1..28: note = source = /note="Description of Artificial Sequence: Synthetic primer"
  source 1..28: mol_type = other DNA
caaatgagcagcctgagagctgaggaca

SEQ ID NO: 122 - DNA, 28 bp, synthetic construct
  misc_feature 1..28: note = source = /note="Description of Artificial Sequence: Synthetic primer"
  source 1..28: mol_type = other DNA
caaatgaacagcctgagagacgaggaca

SEQ ID NO: 123 - DNA, 28 bp, synthetic construct
  misc_feature 1..28: note = source = /note="Description of Artificial Sequence: Synthetic primer"
  source 1..28: mol_type = other DNA
caaatgggcagcctgagagctgaggaca

SEQ ID NO: 124 - DNA, 26 bp, synthetic construct
  misc_feature 1..26: note = source = /note="Description of Artificial Sequence: Synthetic primer"
  source 1..26: mol_type = other DNA
caaatgaacagcctgagagccgggga

SEQ ID NO: 125 - DNA, 28 bp, synthetic construct
  misc_feature 1..28: note = source = /note="Description of Artificial Sequence: Synthetic primer"
  source 1..28: mol_type = other DNA
caaatgaacagtctgagagctgaggaca

SEQ ID NO: 126 - DNA, 28 bp, synthetic construct
  misc_feature 1..28: note = source = /note="Description of Artificial Sequence: Synthetic primer"
  source 1..28: mol_type = other DNA
caaatgagcagtctgagagctgaggaca

SEQ ID NO: 127 - DNA, 20 bp, synthetic construct
  misc_feature 1..20: note = source = /note="Description of Artificial Sequence: Synthetic primer"
  source 1..20: mol_type = other DNA
gccagggggaagaccgatgg

SEQ ID NO: 128 - DNA, 20 bp, synthetic construct
  misc_feature 1..20: note = source = /note="Description of Artificial Sequence: Synthetic primer"
  source 1..20: mol_type = other DNA
gccagggggaagacggatgg

SEQ ID NO: 129 - DNA, 50 bp, synthetic construct
  misc_feature 1..50: note = source = /note="Description of Artificial Sequence: Synthetic primer"
  source 1..50: mol_type = other DNA
aatgatacggcgaccaccgagatctgggaagacgatgggcccttggtgga

SEQ ID NO: 130 - DNA, 31 bp, Homo sapiens
  source 1..31: mol_type = genomic DNA
aggacctgaaaaacgtgttcccacccgaggt

SEQ ID NO: 131 - DNA, 31 bp, Homo sapiens
  source 1..31: mol_type = genomic DNA
aggacctgaacaaggtgttcccacccgaggt

SEQ ID NO: 132 - DNA, 49 bp, Homo sapiens
  source 1..49: mol_type = genomic DNA
cctccaccaagggcccatcggtcttccccctggcgccctgctccaggag

SEQ ID NO: 133 - DNA, 49 bp, Homo sapiens
  source 1..49: mol_type = genomic DNA
cttccaccaagggcccatccgtcttccccctggcgccctgctccaggag

SEQ ID NO: 134 - DNA, 49 bp, Homo sapiens
  source 1..49: mol_type = genomic DNA
cttccaccaagggcccatcggtcttccccctggcgccctgctccaggag

SEQ ID NO: 135 - DNA, 20 bp, synthetic construct
  misc_feature 1..20: note = source = /note="Description of Artificial Sequence: Synthetic primer"
  source 1..20: mol_type = other DNA
agcgacctcgggtgggaaca